European Patent Application EP 4 810 612 A1, published September 23, 2026. Title: 晚疫病抗性基因、生物材料及应用. Applicant: 中国农业科学院深圳农业基因组研究所（岭南现代农业科学与技术广东省实验室深圳分中心）. The sequence listing filed with the application follows.

SEQUENCE LISTING (38 sequences)

SEQ ID NO: 1 - DNA, 4257 bp, Solanum cajamarquense
  source 1..4257: mol_type = genomic DNA; note = Rpi-caj1-C534 genome sequence; note (original language) = Rpi-caj1-C534基因组序列
atggcaaccccacaaacccgttattctttccacgttttcttgagtttcagaggcgaagacacccgaaaaaactttactgatcatctttacacagctctcatcaacgccggaattcgaacttttcgagatgatgacgaaatccgcaggggagaaaacatagaatctgaactgcaaaagggtattcgagaatccaagatttcactagttgtcttctccaaagattacggttcttcaagatggtgtcttgatgagcttgtcaacattcttgatcgaaaaaagaaagagggtcatactgttttgcctgtgttttacactgtgagccctgaggatgtccagaaccaaactggaagttttgctgaagcttttgtgactcatgaaaagagaggaaacgcagagagtggagagaaaagaaaggaatggatggagaagatggagaaatggagagtagctctgaaggaagttgctgaattggaaggaatgtgcttagccaaagaagtagacgggtcagtctcctaaattatccaaacccttggtatttttcttttttttcagtatttgcagttattcccccttcattcattagtcttgagagctatgttagttctaatggtttctggtgaaagaaaatgttgtggcttaataattgctttaatctttactttaagggaaacttggctgatgatattagtgaagtacaatagataataatctaaaactatgttttgttctggattaagtagtcaaccgattgatttcatctatttaaatctggaaattcacttttgaggatcaccgtattccaacttagccaacacacgattctccccaaacaagaaaacctattcatcagttggaaagttctgatgtaaatttgccattcactcagtactagttgtcctgtattttaggttgtggctactgcaatgacatagtgccagtttgctaattcatgagtaaacaagttgtaaacattattttctgagaataacttatagtatctatgcgatgactatcataaatgtccaagtgactaatgtggccggcaaaatcgtctattgtaaaggttatttcaggaaaagatacactggaaatgctaaatgggcaaaatttaaaagatggattgacgaaacttctaccaaggcatgaaaaattaactgtgaacagcccaaactttaaaaagatttaatatgttaaataccctggacagtacgttgagctctaaacaaattcgagcaaaaaagtttaacaaagttggcataaatctaatttgaaagactaatcagatgaaagacacaaagttcaaagctaaagatgataaaaagctacctcaggttggattctagtcaagtgtgacactcacgtgtgagtatgccaaatggcaagtgctatgcataagtcgcgattgaacctcgtggggttcccctaaaagatagagattccgagctttcatgtatattccttttctctgaatgtaatgtattgttggtcatccactctagagacaaacgaggatcgtcttcgggcttcttttgttgctatgaaatgtgtcgtgtgtggatcccattagagaagtctcattactgattattttcaatattttcaacctcaaagactcaaaccactaaaaatagagggtctcttccctattagatctatgctgattttgaaaggagcccacatagacaacatactggcttgtactttatccattataatcacctatatccttaggaaacacattttaatgctcaatatttctggtgattcttcaattagattttgtgtcctcttttccatgaaagtgtgctgccttctaccttggggttatggaggcaccctagttgagctcttgctgtgcgtggatgtgtctgtgctgttttcttttcttttcccttctttccttccttttcctgcttatgtatgccagaagttagtaagacctctctctgactagttgaggtaaaaaacttggacaggacatctagggactcttggaattaaaccctgctctcaaattattctgattaagatagattggagcaataatttcttgctttccacgtaatcttccttcatttctgtgaatgctcttgacttgtatgtgctcttagctattccagtcagcagttcttcaagccattgtgtaattatttgttatcagagtcaaaatgatctatttaaagagtgaaggatatgtaaagggagggtaccaaatagctgaattgacgaatcaaaaggtgcaaaagaacgaaatgttgtcatgatacactccattctccaagtgtggatgcactttgtatcagtatcttttggaagtttttgtatgatatagcctcagttatgatgaggctaaacgtgtccttgtcttaattattttcctaacgggaaatggttcactgtaatatttcatggttctctatttattgtactactactctctttattttgttgtccatttccctctttgttgctcctcaatattgtcaaattcttcacaacacacaagtaaaagtaaatatcactcattttttctcctgtagtaccagtaagccacatatatttcatctttgttgcttttctgggaaatgtaaaagtatattgatttagcattaagagattgctttaaaggtatactttcacgtttttcttaatagtgcctaggcacctaaccaggttattttgtttattgatgattaatatgacagatcatcctggtgtgttatgcttgctctaaatgaagtattaccatatcagtgaactctttttatttgttctccagtacttggcaagttgcagtgctttactgaattttcatcttgttttgtctctaacatttgcactgcatctcaggcatgaggcaaaattcatccaaaagatcatcaaggagatactcaaaagattgaaccgcacagtacttagtgtaccttcatacacagttggattagagtttcgagtgaaggacattaactcatggttacaggatgaatccagtgaagttggcattgggatgatctgtggacttggtggcgttggaaagactactgttgctaaagtagcttacaactctaattatgacagatttgatgggagttgctttcttgcaaatgtcagagaaatctctgagaaacatccaaatggtcaggtttatttgcaaaaacaaatttttgaaagtattttgaaaggcagaaaggaaaaaatatacaatgctgatgaaggaattgtcaaaatgaaagatgctattggcaacaaaaaggtttttattgtatttgatgatgtggatcagctggatgtcttagattcacttattgggacaagggattggttttatccagggagtaaaattctcataacgacaaggtgtgagaaactgttgaagtcctatgagaggcatatgctattcaagatagaggaacttggggatgatgagtctctaaagctcttcagttggtacgcttttgcgcaagaccacccattagaagagttcaagatgctttcaacagaagcaatacagcattgcggtgggcttccattagctctttatgatttgggttcgtttctttcagggagaggtatggaaatatggagaagtaaattgcagaaattagaagcaatccctcatagcagagttcaaaagaatcttgagataagctacaagtctctagatgatcatgaccagaggttgttcctccttattgcttcattatttgttgggaaggacaaagattatgttatcaaatttttagagaacagcgatttgcacccaacagttggaattcagaacctcattgacagatccctcatcagcattgatgacgaaaacaaagtgatgatgcctccacttattcaggacatgggaaaagaaattattcgtcgagaatcaccagatgatcctgagagattgtgtaaattattgaaccaatgtggtctattaaattgcttgacagaaaacaatgtaagaatcttgacttttctatccatgttaagcttgtcttggtagattctcgaagtgttcttgtttctcacagaatctttctgcaacaggaaactgatgcagatggagtagacctcccaggcaaacatctgccagaaggtggtcttgtcccagcacttgaccctaatggtgcaaaaagaccgtattatcaagattttccagaaatagctgttctgccatacctaggtaattcgttgaaaaggcactttgtaggacttctttcgacgttccccttatctggtagcctcaagagattcttcccatga

SEQ ID NO: 2 - DNA, 4258 bp, Solanum cajamarquense
  source 1..4258: mol_type = genomic DNA; note = Rpi-caj1-C813 genome sequence; note (original language) = Rpi-caj1-C813基因组序列
atggcaaccccacaaacccgttattctttccacgttttcttgagtttcagaggcgaagacacccgaaaaaactttactgatcatctttacacagctctcatcaacgccggaattcgaacttttcgagatgatgacgaaatccgcaggggagaaaacatagaatctgaactgcaaaagggtattcgagaatccaagatttcactagttgtcttctccaaagattacggttcttcaagatggtgtcttgatgagcttgtcaacattcttgatcgaaaaaagaaagagggtcatactgttttgcctgtgttttacactgtgagccctgaggatgtccagaaccaaactggaagttttgctgaagcttttgtgactcatgaaaagagaggaaacgcagagagtggagagaaaagaaaggaatggatggagaagatggagaaatggagagtagctctgaaggaagttgctgaattggaaggaatgtgcttagccaaagaagtagacgggtcagtctcctaaattatccaaacccttggtatttttcttctttttcagtatttgcagttattcccccttcattcattagtcttgagagctatgttagttctaatggtttctggtgaaagaaaatgttgtggcttaataattgctttaatctttactttaagggaaacttggctgatgatattagtgaagtacaatagataataatctaaaactatgtttggttctggattaagtagtcaaccgattgatttcatctatttaaatctggaaattcacttttgaggatcacggtattccaacttagccaacacacgattctccccaaacaagaaaacctattcatcagttggaaagttctgatgtaaatttgccattcactcagtactagttgtcctgtattttaggttgtggctactgcaatgacatagtgccagtttgctaattcatgagtaaacaagttgtaaacattattttctgagaataacttatagtatctatgcatctgaccatcataaatgtccaagtgactaatgtggccggcaaaatcgtctattgtaaaggttatttcaggaaaagatacactggaaatgctaaatgggcaaaatttaaaagatggattgacgaaacttctaccaaggcatgaaaaattaactgtgaacagcccaaactttaaaaagatttaatatgttaaataccctggacagtacgttgagctctaaacaaattcgagcaaaaaagtttaacaaagttggcataaatctaatttgaaagactaatcagatgaaagacacaaagttcaaagctaaagatgataaaaagctacctcaggttggattctagtcaagtgtgacactcacgtgtgagtatgccaaatggcaagtgctatgcataagtcacgattgaacctcgtggggttcccctaaaagatagagattccgagctttcatgtatattccttttctctgaatgtaatgtattgttggtcatccactctagagacaaacgaggatcgtcttcgggcttcttttgttgctatgaaatgtgtcgcgtgtggatcccattagagaagtctcattactgattcttttcaatattttcaacctcaaagactcaaaccactaaaaatagagggtctcttccctattagatctatgctgattttgaaaggagcccacatagacaacatactggcttgtactttatccattataatcacctatatccttaggaaacacattttaatgctcaatatttctggtgattcttcaattagattttgtgtcctcttttccatgaatgtgtgctgccttctaccttggggttatggaggcaccctagttgagctcttgctgtgcgtggatgtgtctgtgctgttttcttttcttttcccttctttccttccttttcctgcttatgtatgccagaagttagtaagacctctctctgactagttgaggtaaaaaacttggacaggacatctagggactcttggaattaaaccctgctctcaaattattctgattaagatagattggagcaataatttcttgctttccacgtaatcttccttcatttctgtgaatgctcttgacttgtatgtgctcttagctattccagtcagcagttcttcaagccattgtgtaattatttgttatcagagtcaaaatgatctatttaaagagtgaaggatatgtaaagggagggtaccaaatagctgaattgacgaatcaaaaggtgcaaaagaacgaaatgttgtcatgatacactccattctccaagtgtggatgcactttgtatcagtatcttttggaagtttttgtatgatatagcctcagttatgatgaggctaaacgtgtccttgtcttaattattttcctaacgggaaatggttcactgtaatatttcatggttctctatttattgtactactactctctttattttgctgtccatttccctctttgttgctcctcaatattgtcaaattcttcacaacacacaagtaaaagtaaatatcactcattttttctcctgtagtaccagtaagccacatatatttcatctttgttgcttttctgggaaatgtaaaagtttattgatttagcattaagagattgctttaaaggtatactttcacgtttttcttaatagtgcctaggcacttaaccaggttattttgtttattgatgattaatatgacagatcatcctggtgtgttatgcttgctctaaatgaagtattaccatatcagtgaactctttttatttgttctccagtacttggcaagttgcagtgctttacagaattttcatcttgttttgtctctaacatttgcactgcatctcaggcatgaggcaaaattcatccaaaagatcatcaaggagatactcaaaagattgaaccgcacagtacttagtgtaccttcatacacagttggattagagtttcgagtgaaggacattaactcatggttacaggatgaatccagtgaagttggcattgggatgatctgtggacttggtggtgttggaaagactactgttgctaaagtagcttacaactctaattatgacagatttgatgggagttgctttcttgcaaatgtcagagaaatctctgagaaacatccaaatggtcaggtttatttgcaaaaacaaatttttgaaagtattttgaaaggcagaaaggaaaaaatatacaatgctgatgaaggaattgtcaaaatgaaagatgctattggcaacaaaaaggtttttattgtatttgatgatgtggatcagctggatgtcttagattcacttattgggacaagggattggttttatccagggagtaaaattctcataacgacaaggtgtgagaaactgttgaagtcctatgagaggcatatgctattcaagatagaggaacttggggatgatgagtctctaaagctcttcagttggtacgcttttgcacaagaccacccattagaagagttcaagatgctttcaacagaagcaatacagcattgcggtgggcttccattagctctttatgatttgggttcgtttctttcagggagaggtatggaaatatggagaagtaaattgcagaaattagaagcaatccctcatagcagagttcaaaagaatcttgagataagctacaagtctctagatgatcatgaccagaggttgttcctccttattgcttcattatttgttgggaaggacaaagattatgttatcaaatttttagagaacagcgatttgcacccaacagttggaattcagaacctcattgacagatccctcatcagcattgatgacgaaaacaaagtgatgatgcctccacttattcaggacatgggaaaagaaattattcgtcgagaatcaccagatgatcccgagagattgtgtaaattattgaaccaatgtggtctatcaaattacttgacagaaaacaatgtaagaatcttgacttttctattcatgttaagcttgtcttggtagattctcaaagtgttcttgtttctcacagaatctttctgcaacaggaaactgatgcagatggagtagacctcccaggcaaacatctgccagaaggtggtcttgtcccagcacttgaccctaatggtgcaaaaagaccgtattatcaagattttccagaaatagctgttctgccatacctaggtaattcgttgaaaaggcactttgtaggacttctttcgacgttccccttatctggtagcctcaagagattcttcccatga

SEQ ID NO: 3 - DNA, 4197 bp, Solanum sogarandinum
  source 1..4197: mol_type = genomic DNA; note = Rpi-caj1-C550 genome sequence; note (original language) = Rpi-caj1-C550基因组序列
atggcaaccccacaaacccgttattctttccacgttttcttgagtttcagaggcgaagacacccgaaaaaactttactgatcatctctacacagctctcatcaacgctggaattcgaacttttcgagatgatgacgaaattcgcaggggagaaaacatagaatctgaactgcaaaagggtattcgagaatccaagatttcactagttgtcttctctgaagattacggttcttcaagatggtgtcttgatgagcttgtcaacattcttgatcgaagaaagaaagagggtcatactgttttgcctgtgttttacactgtcagccctgaggatgtccagaaccaaactggaagttttgctaaagcttttgtgaatcatgaaaagagaggaaacgcagagagtggagagaaaagaaaggaatggatggagaagatggagaagtggagagtagctctgaaagaagttgctgaattagaaggaatgtgcttagccaaagaagtagacgggtcagtttcctaaattatccaaacccttggtatttttcttctttttcagtatttgcagttatccccccttcattaattagtgatgagagctatgttagttctaattgtttctggtaaaagaaatagttgtggcttaataattgctttaatgttaacttgaagggaaacttggctgatgatgttagtgatgatctacaactatgttttgttctggattaagtagtcaaccgattaatttcatctatttaaatctggaagttctcttttgaggatcaacggtattccaacttagccaacacacgattctccccaaacaagaaaacctattcatcagttcgaaagttctgatgtaaatttgccattcactcagtactagttgtcctgtattttaggttgtgactattgcaatgacatagtgccagtttgctaattcatgagtaaacaagttgtaaacattattttctgagaataacttatagtatctatgcatctgactatcataaatgtccaagtgactaatgtggcccgcaaaattatctattgtaaaggttatttcaggaaaagatacactggaaatgccaaattaaaagatggattgacgaaacttctaccaaggcatgaaaaattaactgtgaacagcccaaacttaaaagagatttaatatgttaaagaccctggatagtactttgagctctaagcaaattcgagcaaaaaagtttaacaaagttggcataaatctaatttgaaaaactaatcagatgaaaaacacaaagttcaaagctaaagatgataaaaagctacctcaggttggattctagtcaagtgtgacagtcacgtgtgagtatgccaaatggcaagtgctatgcataagtcgcgattgaacctcgtggggttcccctaaaagatagagattcctagctttcatgtatattccttttctctgaatgtaatgtattgtctggcttcttttgttgctatgaaatgtgtcgcgtgtggatcccattagagaagtctcattactgatcctttttcaatattttcaacctcaaagactcaaaccactaaaaatagagggtcttttccctattagatttatgctgattttgaaaggagtccacatagacaacatactgacttgtactttatccatttcaatcacctatatccttaggaaacacattttaatgctcaatatttctggcgactcttcaattagattttgtgtcctcttttccatggatgtgtgctgccttctaccttgggggtatggaggcaccctagttgaactcttgctgtgcgtggatgtgtctgttgttttcttttcttttcccttctttccttccttttcctgtttatcatatgccagaagttagtaagacctctctctgactagttgaggtaaaaaacttggacaagacaactagggactcttggatttaaaccttgctctcaaattattctgattaagatagatgggagcaataatttcttgctttccacgtaatcttccttcatgtctgtgaatgctcgacttgtatgtgcttttagcttttccaatcagcagttcttcaagccattgtgtcctcaattatttgttatcagagtcaaaatgatctatttaaagagtgaaggatatataaagggagggtaccaaatagctgaatagacaaatcaaaaggtacaaaagaacgaaatgttgtcatgatacactccattctccaagtgtggatgcactttgtatcagtatcttttggaaatttttgtatgatatagcctcagttatgatgaggctaaacgtgtccttgtcttaatcattttcctaaccggaaatggttcactgtaatatttcatggttctctatttattgtactactactctctttgttttgctgcccatttccctctttgtttctcctcaatattgtcaaattcttcacagcacacaaattaaagtaaatatcactcattttttctcctgtagtaccagtaagccacatatttcatctttgttgcttttctgggaaatgtagtttattgatttagcattaagagattgctttaaaggtatactttcacgttttttcttaatagtgcctaggcacctaaccaggttattttgtttattgatgattaatatgacagatcatcctggtgtgttgtgcttgctctaaatgaagtattaccatatcagtgaactctctttatttgttctccagtacttggcaagttgcagtgcttaactgaattttcatcttgcttcgtctctaacatttgcactgcatctcaggcatgaggcaaaattcatccaaaagatcatcaaggagatactcaaaagattgaatcgcacagtacttagtgtaccttcatacacagttggattagagtctcgagtgaaggacattaactcatggttacaggatgaatccagtcaagttggcattgggatgatctgtggacttggtggcgttggaaagactactgttgctaaagtagcttacaactctaattatgacagatttgatgggagttgctttcttgcaaatgtcagagaaatctctgagaaacatccaaatggtcaggtttatttgcaaaaacaaatttttgaaagtattttgaaaggcagaaaggaaaaaatatacaatgctgatgaaggaattgtcaaaatgaaagatgctattggcaacaaaaaggtttttattgtatttgatgatgtggatcagctggatgtcttagattcacttattgggacaagggattggttttatccggggagtaaaatactcataacgacaaggtgtgagaaactgttgaagtcttatgagaggcacatgctattcaagattaaggaacttggggatgatgagtctctaaagctcttcagttggtatgcttttgcacaagaccacccattagaagagttcaagatgctttcaacagaagcaatacagcattgcggtgggcttccattagctctttatgatctgggttcgtttctttcagggagacgtatggaaatatggagaagcaaattgcagaaattggaagcaatccctcatagcagagttcaaaagaatcttgagataagctataagtctctagatgatcatgaccagaggttgttcctccttattacttcattatttgttgggaaggacaaagattatgttatcaaatttttagagaacagcgatttgcacccaacagttggaattcagaacctcattgacagatccctcatcagcattgatgacgaaaacaaagtgatgatgcctccacttattcaggacatgggaaaagaaattattcgtcgagaatcaccagatgatcccgagagattgtgtaaattattgaaccaatgtggtctatcaaattgcttgacagaaaacaatgtgagaatcttgacttttctattcatgttaagcttgtcttggtagattctcaaagtgttcttgtttctcacagaatctttctgcaacaggaaactgatgcagatggaatagacctcccaggcacccatctgccagaagatggtcttgtcccagcacttggtcctaatggtgcaaaaagaccatattatcaagattttcctgaaatagctgttctgccatacctaggtaattcgttgaaaaggcgctttgtaggacttctttcgacgttccccttatctggtggcctcaaaagattcttcccatga

SEQ ID NO: 4 - DNA, 4489 bp, Solanum cardiophyllum
  source 1..4489: mol_type = genomic DNA; note = Rpi-caj1-C509 genome sequence; note (original language) = Rpi-caj1-C509基因组序列
cgcaattgccttaacaaacaaacaaacgatataatacctcgtctcccttcccaccccttacaaaaaaacattgtagtgcggacctttccattgacttttaagtcctcaaattttccatttctgttctcaagttttcattgtcaaaatctcaattggatcattatcctctgtctctgcataaactctcagttgggtcatcgttttcttcgacttttttgtatggcaaccccacaaacccgttattctttccacgttttcttgagtttcagaggcgaagacacccggaaaaactttactgatcatctctacacagctctcatcaacgctggaattcgaacttttcgagatgatgacgaaatccgcaggggagaaaacatagaatctgaactgcaaaagggtattcgagaatccaagatttcactagttgtcttctccaaagattacggttcttcaagatggtgtcttgatgaacttgtcaacattcttgatcgaagaaagaaagagggtcatactgttttgcctgtgttttacactgtgagccctgaggatgtccagaaccaaactggaagttttgctgaagcttttgtgaatcatgaaaagagaggaaatgcagagagtggagagaaaagaaaggaatggatggagaagatggacaagtggagagtagctctgaaagaagttgctgaattagaaggaatgtgcttagccaaagaagtagacgggtgagcttcctaaattatccaaacccttggtatttttcttctttttcagtatttgcagttattcccccttcattaattagtcttgagagctatgttagttctaattgtttctggtgaaagaaatagttgtggcttaataattgctttaatttttacttgaaggaaaaattggctgatgatgttagtgaagtaccatagataataatctaaaactatgttttgttctggattaagtagtcaaccgattgatttcatctatttaaatctggaagttctcttttgagaatcaacggtactccaacttagccaacagacgattctccccaaacaaggaaacctattcatcagttggaaagttctgatgtaaatttgcctttcactcagtactagttgtcctgtattttaggttgtgactattgcaatgacatagtgccagtttgctaattcatgagtaaacaagttgtaaacattattttctgagaataactttaagtatctatgcatctgactatcataaatgtccaagtgactaatgtggccagcaaaattatctattgcaaaggttatttcaggaaagatacactggaaatgctaaatgggcaaaatttaaaaggtggattgacgaaacttctaccaaggcatgaaaaattaactgtgaacagcccaaacttaaaagagatttaatatgttaaagaccctggatagtacgttgagctctaagcaaattcgagcaaaaaagtttaacaaagttggcataaatctaatttgaaagactaatcagatgaaagacacaaagttcaaagctaaagatgataaaaagctacctcaggttggattctcgtcaagtgtgatactcacatgtgagtatgccaaatggcaagtgctatgcgaaagtcgcgattgaaactcgtggggttcccctaaaagatagagattctagctttcatgtatgttccttttctctgaatgtaatgaattgttggtcatccactctagagacaaatgaggatggtcttcgggcttcttttgtgctatgaaatgtatcgcgtgtggatcccattagagaagtctcattacttatcccttttcaatattttcaacctcaaagacttaaaccactaaaaatagagggtcttttccctattagacctatgctggttttgaaaggagtccacctagacaacatactgtcttgtactttatccatgacaatcacctatatccttaggaaacacattttaatgctcaatatttctgatgactcttcaattagattttgtgtcctcttttccatggatgtgtgctgccttctaccttgggagtatggaggcaccctagttgaactcgtgctgtgcgtggatgtgtctgtgatgttttcttttcttttcccttttttccttacttttcctgcttatcgccagaagttagtaagacctctctctgactagttgaggtaaaaaacttggacaagacaactagggactcttggatttaaaactgctctcaaataattccgatttaaaactagggactcaaaatgggagcaataatttcttgctttcgatgtaatgttccttcatgtcagtgaatgctcttgacttgtatgtgcttatagcttttccaatcagcagttcttcaggccattgtgtcctcaattatttgttatgagagtcaaaatgatctatttaaagagtgaaggatatataaagggagggtaccaaatagctgaatagacaaatcaaaaggtacaaaagaacaaaatgttgtcatgatacactccattctcctagtgtggatgcactttgtatcagtatcttttggaaatttttgtatgatatagcctcagttatgatgaagctaaactgtgtccttgtcttaatcattttcctaaccggaaatggttcactgtaatatttcatggttctctatttattgtactactactctctttattttactgtccatttccctctttgttgcttctcaatattgtcaaattcttcactgtacacaaataaaagtaaatatcactcattttttctcctgtagtaccagtatgccacatatatttcatctttgctgcttttctgggaaatgtataagtttattgatttagcattaagagattgctttaaaggtatactttcacgttttttcttaattgtgcctaggcacctaaccaggttattttgtttattgatgattaatatgacagatcatcctggtgtgttatgcttgctctaaatgaagtattgccatatcagtgaactctctttatttgctctccagtacttggcaagttgcagtgcttaactgaattttcatcttgctttgtctctaacatttgcactgcatctcaggcatgaggcaaaattcatccaaaagatcatcaaggagatactcaaaagattgaatcgcacagtacttagtgtaccttcatacacagttggattagagtctcgagtgaaggacattaactcatggttacaggatcaatccagtgaagttggcattgggatgatctgtggacttggtggcgttggaaagactactgttgctaaagtagcttacaactctaattatgacagatttgatgggagttgctttcttgcaaatgtcagagaaatctctgagaaacatccaaatggtcaggtttatttgcaaaaacaaatttttgaaagtattttgaaaggcagaaaggaaaaaatatacaatgctgatgaaggaattgtcaaaatgaaagatgctattggcaacaaaaaggtttttattgtatttgatgatgtggatcagctggatgtcttagattcacttattgggacaagggattggttttatccagggagtaaaattctcataacgacaaggtgtgagaaactgttgaagtcctatgagaggcacatgctattcaagataaaggaacttggggttgatgagtctctaaagctcttcagttggtatgcttttgcacaagaccacccattagaagagttcaagatgctttcaacagaagcaatacagcattgcggtgggcttccgttagctctttatgatttgggttcgtttctttcagggagaggtatggaaatatggaggagtaaattgcagaaattggaagcaatccctcatagcagagttcaaaagaatcttgagataagctacaagtctctagatgatcatgaccagaggttgttcctccttattgcttcattatttgttgggaaggacaaagattatgttatcaaatttttagagaacagcgatttgcacccaacagttggaattcagaacctcattgacagatccctcatcagcattgatgacgaaaacaaagtgatgatgcctccacttattcaggacatgggaaaagaaattattcgtcgagaatcaccagatgatcccgagagattgtgtaaattattgaaccaatgtggtctatcaaattgcttgacagaaaacaatgtaagaatcttgacttttctattcatgttaagcttgtcttggtagattctcaaagtgttcttgtttctcacagaatctttctgcaacaggaaattgatgcagatggagtagacctcccaggcacccatctgccagaagatggtcttgtcccagcacttggtcctaatggtgcaaaaagaccatattatcaagattttccagaaatagctgttctgccatacctaggtaattcgttgaaaaggcgctttgtaggacttctttcgacgttccccttatctggtggcctcaaaagattcttcccatga

SEQ ID NO: 5 - DNA, 4266 bp, Solanum piurae
  source 1..4266: mol_type = genomic DNA; note = Rpi-caj1-C450 genome sequence; note (original language) = Rpi-caj1-C450基因组序列
atggcaaccccacaaacccgttattctttccatgttttcttgagtttcagaggcgaagacacccggaaaaactttactgatcatctctacacagctctcatcaacgctggaattcgaacttttagagatgatgacgaaatccgcaggggagaaaacatagaatctgaactgcaaaagggtattcgagaatccaagatttcactagttgtcttctccaaagattacggttcttcaagatggtgtcttgatgagcttgtcaacattcttgatcgaagaaagaaagagggtcatactgttttgcctgtcttttacactgtgagccccgaggatgtccagaaccaaactggaagttttgctgaagcttttgtgaatcatgaaaagagaggaaatgcagagagtggagataaaagaaaggaatggatggagaagatggacaaatggagagtagctctgaaagaagttgctgaattagaaggaatgtgcttagccaaagaagtagacgggtgagtttcctaaattttccaaacccttggtatttttcttctttttcagtatttgcagttattcccccttcattaattagtcatgagagctatgttagttctaattgtttctggtgaaagaaatagttgtggcttaataattgctttaatctttacttgaaggaaacttgactgatgatgttagtgaagtaccatagataataatctaaaactatgttttgttctggattaagtagtcaaccgattgatttcatctatttaaatctggaagttctcttttgaggatcaacggtactccaacttagccaacacacgattctccccaaacaagaaaacctattcatcagttggagagttctgatgtaaatttgcctttcactcagtactagttgtcctgtattttaggttgtgactattgcaatgacatagtgccagtttgctaattcatgagtaaacaagttgtaaacattattttctgagaataacttatagtatctatgcatctgactatcataaatgttcaagtgactaatgtggccggcaaaattatctattgtaaaggttatttcaggaaaagatacactggaaatgctaaatgggcaaaatttaaaagatggattgacgaaacttctaccaaggcatgaaaaattaactgtgaacagcccaaacttaaaaaagatttaatatgttaaataccctggatagtacgttgagctctaaacaaattcgagcaaaaaagtttaacaaagttggcataaatctaatttgaaagactaatcagatgaaagacacaaagttcaaagctaaagatgataaaaagctacctcaggttggattctagtcaagtgtgacactcacgtgtgagtatgccaaatggcaagtgctatgcataagtcgcgattgaacctcgtggggttcccctaaaagatagagattccttgctttcatgtatattccttttctctgaatgtaatgtattgttggtcagtcactctagagacgaacgaggatggtcttctggcttcttttgttgctatgaaatgtgtcgcatgtggatcccattggagaagtctcattactgatcctttttcaatattttcaacctcaaagactcaaaccactaaaaatagaatgtcttttccctattagatctgctgatttttaaaggagtccacatagacaacatactgacctgtactttatccattacaatcatctatatccttaggaaacacattttaatgctcaacatttctggcgactcttcaattagattttgtgtcctcttttccatgaatgtgtgctgccttctaccttgggggtatggaggcaccctagttgaactcttgctgtgtgtggatgatgtgtctgtgctgttttcttttcttttcccttctttccttccttttcctgcttatcatatgccagaagttagtaagacctctgtctgactagttgaggtaaaaaacttggacaaggcaactagggactcttggatttaaaacttgctctcaaattattccgattaagatagatgggagcaataatttcttgctttccatgtaatcttccttcatgtctgtgaatgctcttgacttgtatgtgcttttagcttttccaatcagcagttcttcaagccattgtgtcctcaattatttgttatgagagtcaaaatgatctatttaaagagtgaaggatataaagggagggtaccaaatagctgaatagacaaatcaaaaggtacaaaagaacgaaatgttgtcatgatacactccattctcctagtgtggatgcactttgtatcagtatcttttggaaatttttgtatgatatagcctcagttatgatgaagctaaactgtgtccttgtcttaatcattttcctaaccggaaatggttcactgtaatatttcatggttctctatttattgtactactactctctttattttgctgtccatttccctctttgttgctcctcaatattgtcaaattcttcacagcacacaaataaaagtaaatatcactcattttttctcctgtagtaccagtaagccacatatatttcatctttgttgcttttctgggaaatgtataagtttattgatttagcattaagagattgctttaaaggtatactttcacgttttctcttaattgtgcctaggcacctaaccaggttacttcgtgtattgatgattaatatgacagatcatcctggtgtgttatgcttgctctaaatgaagtattaccatatcagtgaactctttttatttgttctccagtacttggcaagttgcagtgcttaactgaattttcgtcttgcttcgtctctaacatttgcactgcatctcaggcatgaggcaaaattcatccagaagatcatcaaggagatactcaaaagattgaatcgcacagtacttagtgtaccttcatacacagttggattagagtctcgagtgaaggacattaactcatggttacaggatgaatccagtgaagttggcattgggatgatctgtggacttggtggcgttggaaagactactgttgctaaagtagcttacaactctaattatgacagatttgatgggagttgctttcttgccaatgtcagagaaatctctgagaaacatccaaatggtcaggtttatttgcaaaaacaaatttttgaaagtattttgaaaggcagaaaggaaaaaatatacaatgctgatgaaggaattgtcaaaatgaaagatgctattggcaacaaaaaagtttttattgtatttgatgatgtagatcagctggatgtcttagattcacttattgggacaagggattggttttatccggggagtaaaattctcataacaacaaggtgtgagaaactgttgaagtcctatgagaggcacatgctattcaagataaaggaacttggggttgatgagtctctaaagctcttcagttggtatgcttttgcacaagaccacccattagaagagttcaagatgctttcaacagaagcaatacagcattgtggtgggcttccattagctctttatgatttgggttcgtttctttcagggagagatatggaaatatggagaagcaaattgcagaaattggaagcaatccctcatagcagagttcaaaagaatcttgagataagctacaagtctctagatgatcatgaccagaggttgttcctccttattgcttcattatttgttgggaaggacaaagattatgttatcaaatttttagagaacagcgatttgcacccaacagttggaattcagaacctcattgacagatccctcatcagcattgatgacgaaaacaaagtgatgatgcctccacttattcaggacatgggaaaagaaattattcgtcgagaatcaccagatgatcccgagagattgtgtaaattattgaaccaatgtggtctatcaaattgcttgacagaaaacaatgtaagaatcttgacttttctattcatgttaagcttgtcttggtagattctcaaagtgttcttgtttctcacagaatctttttgcaacaggaaactgatgcagatggagtagacctcccaggcacccatctgccagaagatggtcttgtcccagcacttggccctaatggtgcaaaaagaccatattatcaagattttccagaaatagctgttctaccatacctaggtaattcgttgaaaaggcgctttgtaggacttctttcgacgttccccttatctggtggcctcaaaagattcttcccatgat

SEQ ID NO: 6 - DNA, 4508 bp, Solanum candolleanum
  source 1..4508: mol_type = genomic DNA; note = Rpi-caj1-C419 genome sequence; note (original language) = Rpi-caj1-C419基因组序列
atggcaaccccacaaacccgttattctttccacgttttcttgagtttcagaggtgaagacacccgaaaaaactttactgatcatctctacacagctctcatcaacgctggaattcgaacttttcgagatgatgacgaaatccgcaggggagaaaacatagaatctgaactgcaaaagggtattcgagaatccaagatttcactagttgtcttctccgaagattacggttcttcaagatggtgtcttgatgagcttgtcaacattcttaatcgaagaaagaaagagggtcatactgttttacctgtcttttacactgtgagccctgaggatgtccagaaccaaactggaagttttgctaaagcttttgtgaatcatgaaaagagaggaaacgcagagagtggagagaaaagaaaggaatggatggagaagatggagaaatggagagtagctctgaaggaagttgctgaattggaaggaatgtgcttagccaaagaagtagacgggtcagtttcctaaattatccaaacccttggtatttttcttctttttcagtatttgcagttattcccccttcagtaattagtcatgagagctatgttagttctaattgtttctggtgaaagaaatagttatggcttaataattgctttaatctttacttgaagggaaacttggctgatgatattagtgaagtaccatagataataatctaaaactatgttttgttctggattaagtagtcaaccgattgatttcatctatttaaatctggaaattcgcttttgaggatcaacggtattccaacttagccaacacacgattctccccaaacaagaaaacctattcatcagttggaaagttctgatgtaaatttgccattcactcagtactagttgtcctgtattttaggttgtggctattgcaatgacatagtgccagttttctaattcatgagcaaacaagttgtaaacattattttctgagaataatttatagtatctatgcatctgactatcataaatgtccaagtgactggccctcaaagttttctattgtaaaggttatttcaggaaaagatacaatggaaatgctaaatgggcaaaatttaaaagatggatcgacgaaaattctaccaaggcatgaaaaattaactgtgaacagcccaaacttaaagagatttaatatgttaaagaccctggatagtacgttgagctctaagcaaattcgagcaaaaaagtttaacaaagttggcataaatctaatttgaaagactaatcagatgaaagacacaaagttcaaagctaaagatgataaaaagctacctcaggttggattctagtaaagtgtgacagtcacgtgtgagtatgccaaatggcaagtgctatgcataagtcgcgattgaacctcatggggttcccctaaaagatagagattcctagctttcatgtatattccttttctctgaatgtaatgtattgttggttatccactctagagacaaacgaggatggtcttctggcttcttttgttgctatgaaatgtgtcgcatgtggatcccattggagaagtctcattactgatcttttttcaatattttcaacctcaaagactcaaaccactaaaaatagaatgtcttttccctattagatctgctgatttttaaaggagtccacatagaaacatactgacttgtactttatccattacaatcacctatatccttaggaaacacattttaatgctcaatatttttggcgactcttcaattagattttgtgtcctcttttccatgaatgtgtgctgccttctatcttgggggtatggaggcaccctagttgaactcttgctgtgcgtggatgtgtctgtgctgttttcttttcttttcccttctttccttccttttcctgcttatcatatgccagaagttagtaagacctctctctgactagttgaggtaaaaaacttggacaagacaactaggtactcttggatttaaaacttgctctcaaattattccgattaagatagatgggagcaataatttcttgctttccatgtaatcttccttcatgtctgtgaatgctcttgacttgtatgtgcttttagcttttccaatcagcagttcttcaagccattgtgtcctcaattatttgttatgagagtcaaaatgatctatttaaagagtgaaggatatataaagggagggtaccaaatagctgaatagacaaatcaaaaggtacaaaagaacgaaatgttgtcatgatacactccattctcctagtgtggatgcactttgtatcagtaacttttggaaatttttgtatgatatagcctcagttatgatgaagctaaactgtgtccttgtcttaatcattttcctaaccggaaatggttcactgtaatatttcatggttctctatttattgtactactactctctttattttgctgtccatttccctttgttgctcctcaatattgtcaaattcttcacagcacacaaataaaggtaaatatcactcattttttctcctgtagtaccagtaagccacatatatttcatctttgttgcttttctgggaaatgtataagtttttttttttttttggatgacaagggaaacccgcagccgctaccctttgggtgcgcacagggtaaaacccccgctcctatgcaatagctcgcaaaccacataggagaggtaacccgcactaggcaagcctggtgcgacgagctcgacccagaaggcaaaccccttgcttttgctggcaaggggtttcgaacttgagacctccaacatggaagtcccaagcccaaaccactgggccaccccgaagggtgtataagtttattgatttagcattaagagattgctttaaaggtatactttcacgttttttcttaattgtgcctaggcacctaaccaggttatttcgtttattgatgattaatatgacagatcatcctggtgtgttatgcttgctctaatgaagtattgccatatcagtgctctctttatttgttctccagtacttggcaagttgcagtgcttaactgaattttcatcttgctttgtctctaacatttgcactgcatcccaggcatgaggcaaaattcatccaaaagatcatcaaggagatactcaaaagattgaatcgcacagtacttagtgtaccttcatacacagttggattagagtctcgagtgaaggacattaactcatggttacaggatgaatccagtgaagttggcattgggatgatctgtggacttggtggcattggaaagactactgttgctaaagtagcttacaactctaattatgacagatttgatgggagttgctttcttgcaaatgtcagagaaatctctgagaaacatccaaatggtcaggtttatttgcaaaaacaaatttttgaaagtattttgaaaggcagaaaggacaaaatatacaatgctgatgaaggaattgtcaaaatgaaagatgctattggcaacaaaaaggtttttattgtatttgatgatgtggatcagctggatgtcttggattcacttattgggacaagggattggttttatcctgggagtaaaattctcataacgacaaggtgtgagaaactgttgaagtcctatgagaggcacatgctattcaagataaaggaacttggggttgatgagtctctaaagctcttcagttggtatgcttttgcacaagactacccattagaagagttcaagatgctttcaacagaagcaatacagcattgcggtgggcttccgttagctctttatgatttgggttcgtttctttcagggagaggtatggaaatatggaggagtaaattgcagaaattggaagcaatccctcatagcagagttcaaaagaatcttgagataagctacaagtctctagatgatcatgaccagaggttgttccttcttattgcttcattatttgttgggaaggacaaagattatgttatcaaatttttagagaacagtgatttgcacccaacagttggaattcagaacctcattgacagatctctcatcagcattgatgacgaaaacaaagtgatgatgcctccacttattcaggacatgggaaaagaaattattcgtcgagaatcaccagatgatccggagagattgtgtaaattattgaaccaatgtggtctatcaaattgcttgacagaaaacaatgtaagaatcttgacttttctattcatgttaagcttgtcttggtagattctcaaagtgttcttgtttctcacagaatctttgtgcaacaggaaactgatgcagatggagtagacctcccaggcacccatctgccagaagatggtcttgtcccagcacttggtcctaatggtgcaaaaagaccatattatcaagattttccagaaatagctgttctgccatacctaggtaattcgttgaaaaggcgctttgtaggacttctttctacgttccccttatctggtggcctcaaaagattcttcccatga

SEQ ID NO: 7 - protein, 606 aa, Solanum cajamarquense
  source 1..606: note = Rpi-caj1-C534 protein sequence; note (original language) = Rpi-caj1-C534 蛋白质序列
MATPQTRYSFHVFLSFRGEDTRKNFTDHLYTALINAGIRTFRDDDEIRRGENIESELQKGIRESKISLVVFSKDYGSSRWCLDELVNILDRKKKEGHTVLPVFYTVSPEDVQNQTGSFAEAFVTHEKRGNAESGEKRKEWMEKMEKWRVALKEVAELEGMCLAKEVDGHEAKFIQKIIKEILKRLNRTVLSVPSYTVGLEFRVKDINSWLQDESSEVGIGMICGLGGVGKTTVAKVAYNSNYDRFDGSCFLANVREISEKHPNGQVYLQKQIFESILKGRKEKIYNADEGIVKMKDAIGNKKVFIVFDDVDQLDVLDSLIGTRDWFYPGSKILITTRCEKLLKSYERHMLFKIEELGDDESLKLFSWYAFAQDHPLEEFKMLSTEAIQHCGGLPLALYDLGSFLSGRGMEIWRSKLQKLEAIPHSRVQKNLEISYKSLDDHDQRLFLLIASLFVGKDKDYVIKFLENSDLHPTVGIQNLIDRSLISIDDENKVMMPPLIQDMGKEIIRRESPDDPERLCKLLNQCGLLNCLTENNETDADGVDLPGKHLPEGGLVPALDPNGAKRPYYQDFPEIAVLPYLGNSLKRHFVGLLSTFPLSGSLKRFFP

SEQ ID NO: 8 - protein, 606 aa, Solanum cajamarquense
  source 1..606: note = Rpi-caj1-C813 protein sequence; note (original language) = Rpi-caj1-C813蛋白质序列
MATPQTRYSFHVFLSFRGEDTRKNFTDHLYTALINAGIRTFRDDDEIRRGENIESELQKGIRESKISLVVFSKDYGSSRWCLDELVNILDRKKKEGHTVLPVFYTVSPEDVQNQTGSFAEAFVTHEKRGNAESGEKRKEWMEKMEKWRVALKEVAELEGMCLAKEVDGHEAKFIQKIIKEILKRLNRTVLSVPSYTVGLEFRVKDINSWLQDESSEVGIGMICGLGGVGKTTVAKVAYNSNYDRFDGSCFLANVREISEKHPNGQVYLQKQIFESILKGRKEKIYNADEGIVKMKDAIGNKKVFIVFDDVDQLDVLDSLIGTRDWFYPGSKILITTRCEKLLKSYERHMLFKIEELGDDESLKLFSWYAFAQDHPLEEFKMLSTEAIQHCGGLPLALYDLGSFLSGRGMEIWRSKLQKLEAIPHSRVQKNLEISYKSLDDHDQRLFLLIASLFVGKDKDYVIKFLENSDLHPTVGIQNLIDRSLISIDDENKVMMPPLIQDMGKEIIRRESPDDPERLCKLLNQCGLSNYLTENNETDADGVDLPGKHLPEGGLVPALDPNGAKRPYYQDFPEIAVLPYLGNSLKRHFVGLLSTFPLSGSLKRFFP

SEQ ID NO: 9 - protein, 606 aa, Solanum sogarandinum
  source 1..606: note = Rpi-caj1-C550 protein sequence; note (original language) = Rpi-caj1-C550蛋白质序列
MATPQTRYSFHVFLSFRGEDTRKNFTDHLYTALINAGIRTFRDDDEIRRGENIESELQKGIRESKISLVVFSEDYGSSRWCLDELVNILDRRKKEGHTVLPVFYTVSPEDVQNQTGSFAKAFVNHEKRGNAESGEKRKEWMEKMEKWRVALKEVAELEGMCLAKEVDGHEAKFIQKIIKEILKRLNRTVLSVPSYTVGLESRVKDINSWLQDESSQVGIGMICGLGGVGKTTVAKVAYNSNYDRFDGSCFLANVREISEKHPNGQVYLQKQIFESILKGRKEKIYNADEGIVKMKDAIGNKKVFIVFDDVDQLDVLDSLIGTRDWFYPGSKILITTRCEKLLKSYERHMLFKIKELGDDESLKLFSWYAFAQDHPLEEFKMLSTEAIQHCGGLPLALYDLGSFLSGRRMEIWRSKLQKLEAIPHSRVQKNLEISYKSLDDHDQRLFLLITSLFVGKDKDYVIKFLENSDLHPTVGIQNLIDRSLISIDDENKVMMPPLIQDMGKEIIRRESPDDPERLCKLLNQCGLSNCLTENNETDADGIDLPGTHLPEDGLVPALGPNGAKRPYYQDFPEIAVLPYLGNSLKRRFVGLLSTFPLSGGLKRFFP

SEQ ID NO: 10 - protein, 679 aa, Solanum cardiophyllum
  source 1..679: note = Rpi-caj1-C509 protein sequence; note (original language) = Rpi-caj1-C509蛋白质序列
RNCLNKQTNDIIPRLPSHPLQKNIVVRTFPLTFKSSNFPFLFSSFHCQNLNWIIILCLCINSQLGHRFLRLFCMATPQTRYSFHVFLSFRGEDTRKNFTDHLYTALINAGIRTFRDDDEIRRGENIESELQKGIRESKISLVVFSKDYGSSRWCLDELVNILDRRKKEGHTVLPVFYTVSPEDVQNQTGSFAEAFVNHEKRGNAESGEKRKEWMEKMDKWRVALKEVAELEGMCLAKEVDGHEAKFIQKIIKEILKRLNRTVLSVPSYTVGLESRVKDINSWLQDQSSEVGIGMICGLGGVGKTTVAKVAYNSNYDRFDGSCFLANVREISEKHPNGQVYLQKQIFESILKGRKEKIYNADEGIVKMKDAIGNKKVFIVFDDVDQLDVLDSLIGTRDWFYPGSKILITTRCEKLLKSYERHMLFKIKELGVDESLKLFSWYAFAQDHPLEEFKMLSTEAIQHCGGLPLALYDLGSFLSGRGMEIWRSKLQKLEAIPHSRVQKNLEISYKSLDDHDQRLFLLIASLFVGKDKDYVIKFLENSDLHPTVGIQNLIDRSLISIDDENKVMMPPLIQDMGKEIIRRESPDDPERLCKLLNQCGLSNCLTENNEIDADGVDLPGTHLPEDGLVPALGPNGAKRPYYQDFPEIAVLPYLGNSLKRRFVGLLSTFPLSGGLKRFFP

SEQ ID NO: 11 - protein, 606 aa, Solanum piurae
  source 1..606: note = Rpi-caj1-C450 protein sequence; note (original language) = Rpi-caj1-C450蛋白质序列
MATPQTRYSFHVFLSFRGEDTRKNFTDHLYTALINAGIRTFRDDDEIRRGENIESELQKGIRESKISLVVFSKDYGSSRWCLDELVNILDRRKKEGHTVLPVFYTVSPEDVQNQTGSFAEAFVNHEKRGNAESGDKRKEWMEKMDKWRVALKEVAELEGMCLAKEVDGHEAKFIQKIIKEILKRLNRTVLSVPSYTVGLESRVKDINSWLQDESSEVGIGMICGLGGVGKTTVAKVAYNSNYDRFDGSCFLANVREISEKHPNGQVYLQKQIFESILKGRKEKIYNADEGIVKMKDAIGNKKVFIVFDDVDQLDVLDSLIGTRDWFYPGSKILITTRCEKLLKSYERHMLFKIKELGVDESLKLFSWYAFAQDHPLEEFKMLSTEAIQHCGGLPLALYDLGSFLSGRDMEIWRSKLQKLEAIPHSRVQKNLEISYKSLDDHDQRLFLLIASLFVGKDKDYVIKFLENSDLHPTVGIQNLIDRSLISIDDENKVMMPPLIQDMGKEIIRRESPDDPERLCKLLNQCGLSNCLTENNETDADGVDLPGTHLPEDGLVPALGPNGAKRPYYQDFPEIAVLPYLGNSLKRRFVGLLSTFPLSGGLKRFFP

SEQ ID NO: 12 - protein, 606 aa, Solanum candolleanum
  source 1..606: note = Rpi-caj1-C419 protein sequence; note (original language) = Rpi-caj1-C419蛋白质序列
MATPQTRYSFHVFLSFRGEDTRKNFTDHLYTALINAGIRTFRDDDEIRRGENIESELQKGIRESKISLVVFSEDYGSSRWCLDELVNILNRRKKEGHTVLPVFYTVSPEDVQNQTGSFAKAFVNHEKRGNAESGEKRKEWMEKMEKWRVALKEVAELEGMCLAKEVDGHEAKFIQKIIKEILKRLNRTVLSVPSYTVGLESRVKDINSWLQDESSEVGIGMICGLGGIGKTTVAKVAYNSNYDRFDGSCFLANVREISEKHPNGQVYLQKQIFESILKGRKDKIYNADEGIVKMKDAIGNKKVFIVFDDVDQLDVLDSLIGTRDWFYPGSKILITTRCEKLLKSYERHMLFKIKELGVDESLKLFSWYAFAQDYPLEEFKMLSTEAIQHCGGLPLALYDLGSFLSGRGMEIWRSKLQKLEAIPHSRVQKNLEISYKSLDDHDQRLFLLIASLFVGKDKDYVIKFLENSDLHPTVGIQNLIDRSLISIDDENKVMMPPLIQDMGKEIIRRESPDDPERLCKLLNQCGLSNCLTENNETDADGVDLPGTHLPEDGLVPALGPNGAKRPYYQDFPEIAVLPYLGNSLKRRFVGLLSTFPLSGGLKRFFP

SEQ ID NO: 13 - DNA, 1821 bp, Solanum cajamarquense
  source 1..1821: mol_type = other DNA; note = Rpi-caj1-C534 coding DNA sequence; note (original language) = Rpi-caj1-C534 CDS序列
atggcaaccccacaaacccgttattctttccacgttttcttgagtttcagaggcgaagacacccgaaaaaactttactgatcatctttacacagctctcatcaacgccggaattcgaacttttcgagatgatgacgaaatccgcaggggagaaaacatagaatctgaactgcaaaagggtattcgagaatccaagatttcactagttgtcttctccaaagattacggttcttcaagatggtgtcttgatgagcttgtcaacattcttgatcgaaaaaagaaagagggtcatactgttttgcctgtgttttacactgtgagccctgaggatgtccagaaccaaactggaagttttgctgaagcttttgtgactcatgaaaagagaggaaacgcagagagtggagagaaaagaaaggaatggatggagaagatggagaaatggagagtagctctgaaggaagttgctgaattggaaggaatgtgcttagccaaagaagtagacgggcatgaggcaaaattcatccaaaagatcatcaaggagatactcaaaagattgaaccgcacagtacttagtgtaccttcatacacagttggattagagtttcgagtgaaggacattaactcatggttacaggatgaatccagtgaagttggcattgggatgatctgtggacttggtggcgttggaaagactactgttgctaaagtagcttacaactctaattatgacagatttgatgggagttgctttcttgcaaatgtcagagaaatctctgagaaacatccaaatggtcaggtttatttgcaaaaacaaatttttgaaagtattttgaaaggcagaaaggaaaaaatatacaatgctgatgaaggaattgtcaaaatgaaagatgctattggcaacaaaaaggtttttattgtatttgatgatgtggatcagctggatgtcttagattcacttattgggacaagggattggttttatccagggagtaaaattctcataacgacaaggtgtgagaaactgttgaagtcctatgagaggcatatgctattcaagatagaggaacttggggatgatgagtctctaaagctcttcagttggtacgcttttgcgcaagaccacccattagaagagttcaagatgctttcaacagaagcaatacagcattgcggtgggcttccattagctctttatgatttgggttcgtttctttcagggagaggtatggaaatatggagaagtaaattgcagaaattagaagcaatccctcatagcagagttcaaaagaatcttgagataagctacaagtctctagatgatcatgaccagaggttgttcctccttattgcttcattatttgttgggaaggacaaagattatgttatcaaatttttagagaacagcgatttgcacccaacagttggaattcagaacctcattgacagatccctcatcagcattgatgacgaaaacaaagtgatgatgcctccacttattcaggacatgggaaaagaaattattcgtcgagaatcaccagatgatcctgagagattgtgtaaattattgaaccaatgtggtctattaaattgcttgacagaaaacaatgaaactgatgcagatggagtagacctcccaggcaaacatctgccagaaggtggtcttgtcccagcacttgaccctaatggtgcaaaaagaccgtattatcaagattttccagaaatagctgttctgccatacctaggtaattcgttgaaaaggcactttgtaggacttctttcgacgttccccttatctggtagcctcaagagattcttcccatga

SEQ ID NO: 14 - DNA, 1821 bp, Solanum cajamarquense
  source 1..1821: mol_type = other DNA; note = Rpi-caj1-C813 coding DNA sequence; note (original language) = Rpi-caj1-C813 CDS序列
atggcaaccccacaaacccgttattctttccacgttttcttgagtttcagaggcgaagacacccgaaaaaactttactgatcatctttacacagctctcatcaacgccggaattcgaacttttcgagatgatgacgaaatccgcaggggagaaaacatagaatctgaactgcaaaagggtattcgagaatccaagatttcactagttgtcttctccaaagattacggttcttcaagatggtgtcttgatgagcttgtcaacattcttgatcgaaaaaagaaagagggtcatactgttttgcctgtgttttacactgtgagccctgaggatgtccagaaccaaactggaagttttgctgaagcttttgtgactcatgaaaagagaggaaacgcagagagtggagagaaaagaaaggaatggatggagaagatggagaaatggagagtagctctgaaggaagttgctgaattggaaggaatgtgcttagccaaagaagtagacgggcatgaggcaaaattcatccaaaagatcatcaaggagatactcaaaagattgaaccgcacagtacttagtgtaccttcatacacagttggattagagtttcgagtgaaggacattaactcatggttacaggatgaatccagtgaagttggcattgggatgatctgtggacttggtggtgttggaaagactactgttgctaaagtagcttacaactctaattatgacagatttgatgggagttgctttcttgcaaatgtcagagaaatctctgagaaacatccaaatggtcaggtttatttgcaaaaacaaatttttgaaagtattttgaaaggcagaaaggaaaaaatatacaatgctgatgaaggaattgtcaaaatgaaagatgctattggcaacaaaaaggtttttattgtatttgatgatgtggatcagctggatgtcttagattcacttattgggacaagggattggttttatccagggagtaaaattctcataacgacaaggtgtgagaaactgttgaagtcctatgagaggcatatgctattcaagatagaggaacttggggatgatgagtctctaaagctcttcagttggtacgcttttgcacaagaccacccattagaagagttcaagatgctttcaacagaagcaatacagcattgcggtgggcttccattagctctttatgatttgggttcgtttctttcagggagaggtatggaaatatggagaagtaaattgcagaaattagaagcaatccctcatagcagagttcaaaagaatcttgagataagctacaagtctctagatgatcatgaccagaggttgttcctccttattgcttcattatttgttgggaaggacaaagattatgttatcaaatttttagagaacagcgatttgcacccaacagttggaattcagaacctcattgacagatccctcatcagcattgatgacgaaaacaaagtgatgatgcctccacttattcaggacatgggaaaagaaattattcgtcgagaatcaccagatgatcccgagagattgtgtaaattattgaaccaatgtggtctatcaaattacttgacagaaaacaatgaaactgatgcagatggagtagacctcccaggcaaacatctgccagaaggtggtcttgtcccagcacttgaccctaatggtgcaaaaagaccgtattatcaagattttccagaaatagctgttctgccatacctaggtaattcgttgaaaaggcactttgtaggacttctttcgacgttccccttatctggtagcctcaagagattcttcccatga

SEQ ID NO: 15 - DNA, 1821 bp, Solanum sogarandinum
  source 1..1821: mol_type = other DNA; note = Rpi-caj1-C550 coding DNA sequence; note (original language) = Rpi-caj1-C550 CDS序列
atggcaaccccacaaacccgttattctttccacgttttcttgagtttcagaggcgaagacacccgaaaaaactttactgatcatctctacacagctctcatcaacgctggaattcgaacttttcgagatgatgacgaaattcgcaggggagaaaacatagaatctgaactgcaaaagggtattcgagaatccaagatttcactagttgtcttctctgaagattacggttcttcaagatggtgtcttgatgagcttgtcaacattcttgatcgaagaaagaaagagggtcatactgttttgcctgtgttttacactgtcagccctgaggatgtccagaaccaaactggaagttttgctaaagcttttgtgaatcatgaaaagagaggaaacgcagagagtggagagaaaagaaaggaatggatggagaagatggagaagtggagagtagctctgaaagaagttgctgaattagaaggaatgtgcttagccaaagaagtagacgggcatgaggcaaaattcatccaaaagatcatcaaggagatactcaaaagattgaatcgcacagtacttagtgtaccttcatacacagttggattagagtctcgagtgaaggacattaactcatggttacaggatgaatccagtcaagttggcattgggatgatctgtggacttggtggcgttggaaagactactgttgctaaagtagcttacaactctaattatgacagatttgatgggagttgctttcttgcaaatgtcagagaaatctctgagaaacatccaaatggtcaggtttatttgcaaaaacaaatttttgaaagtattttgaaaggcagaaaggaaaaaatatacaatgctgatgaaggaattgtcaaaatgaaagatgctattggcaacaaaaaggtttttattgtatttgatgatgtggatcagctggatgtcttagattcacttattgggacaagggattggttttatccggggagtaaaatactcataacgacaaggtgtgagaaactgttgaagtcttatgagaggcacatgctattcaagattaaggaacttggggatgatgagtctctaaagctcttcagttggtatgcttttgcacaagaccacccattagaagagttcaagatgctttcaacagaagcaatacagcattgcggtgggcttccattagctctttatgatctgggttcgtttctttcagggagacgtatggaaatatggagaagcaaattgcagaaattggaagcaatccctcatagcagagttcaaaagaatcttgagataagctataagtctctagatgatcatgaccagaggttgttcctccttattacttcattatttgttgggaaggacaaagattatgttatcaaatttttagagaacagcgatttgcacccaacagttggaattcagaacctcattgacagatccctcatcagcattgatgacgaaaacaaagtgatgatgcctccacttattcaggacatgggaaaagaaattattcgtcgagaatcaccagatgatcccgagagattgtgtaaattattgaaccaatgtggtctatcaaattgcttgacagaaaacaatgaaactgatgcagatggaatagacctcccaggcacccatctgccagaagatggtcttgtcccagcacttggtcctaatggtgcaaaaagaccatattatcaagattttcctgaaatagctgttctgccatacctaggtaattcgttgaaaaggcgctttgtaggacttctttcgacgttccccttatctggtggcctcaaaagattcttcccatga

SEQ ID NO: 16 - DNA, 2040 bp, Solanum cardiophyllum
  source 1..2040: mol_type = other DNA; note = Rpi-caj1-C509 coding DNA sequence; note (original language) = Rpi-caj1-C509 CDS序列
cgcaattgccttaacaaacaaacaaacgatataatacctcgtctcccttcccaccccttacaaaaaaacattgtagtgcggacctttccattgacttttaagtcctcaaattttccatttctgttctcaagttttcattgtcaaaatctcaattggatcattatcctctgtctctgcataaactctcagttgggtcatcgttttcttcgacttttttgtatggcaaccccacaaacccgttattctttccacgttttcttgagtttcagaggcgaagacacccggaaaaactttactgatcatctctacacagctctcatcaacgctggaattcgaacttttcgagatgatgacgaaatccgcaggggagaaaacatagaatctgaactgcaaaagggtattcgagaatccaagatttcactagttgtcttctccaaagattacggttcttcaagatggtgtcttgatgaacttgtcaacattcttgatcgaagaaagaaagagggtcatactgttttgcctgtgttttacactgtgagccctgaggatgtccagaaccaaactggaagttttgctgaagcttttgtgaatcatgaaaagagaggaaatgcagagagtggagagaaaagaaaggaatggatggagaagatggacaagtggagagtagctctgaaagaagttgctgaattagaaggaatgtgcttagccaaagaagtagacgggcatgaggcaaaattcatccaaaagatcatcaaggagatactcaaaagattgaatcgcacagtacttagtgtaccttcatacacagttggattagagtctcgagtgaaggacattaactcatggttacaggatcaatccagtgaagttggcattgggatgatctgtggacttggtggcgttggaaagactactgttgctaaagtagcttacaactctaattatgacagatttgatgggagttgctttcttgcaaatgtcagagaaatctctgagaaacatccaaatggtcaggtttatttgcaaaaacaaatttttgaaagtattttgaaaggcagaaaggaaaaaatatacaatgctgatgaaggaattgtcaaaatgaaagatgctattggcaacaaaaaggtttttattgtatttgatgatgtggatcagctggatgtcttagattcacttattgggacaagggattggttttatccagggagtaaaattctcataacgacaaggtgtgagaaactgttgaagtcctatgagaggcacatgctattcaagataaaggaacttggggttgatgagtctctaaagctcttcagttggtatgcttttgcacaagaccacccattagaagagttcaagatgctttcaacagaagcaatacagcattgcggtgggcttccgttagctctttatgatttgggttcgtttctttcagggagaggtatggaaatatggaggagtaaattgcagaaattggaagcaatccctcatagcagagttcaaaagaatcttgagataagctacaagtctctagatgatcatgaccagaggttgttcctccttattgcttcattatttgttgggaaggacaaagattatgttatcaaatttttagagaacagcgatttgcacccaacagttggaattcagaacctcattgacagatccctcatcagcattgatgacgaaaacaaagtgatgatgcctccacttattcaggacatgggaaaagaaattattcgtcgagaatcaccagatgatcccgagagattgtgtaaattattgaaccaatgtggtctatcaaattgcttgacagaaaacaatgaaattgatgcagatggagtagacctcccaggcacccatctgccagaagatggtcttgtcccagcacttggtcctaatggtgcaaaaagaccatattatcaagattttccagaaatagctgttctgccatacctaggtaattcgttgaaaaggcgctttgtaggacttctttcgacgttccccttatctggtggcctcaaaagattcttcccatga

SEQ ID NO: 17 - DNA, 1821 bp, Solanum piurae
  source 1..1821: mol_type = other DNA; note = Rpi-caj1-C450 coding DNA sequence; note (original language) = Rpi-caj1-C450 CDS序列
atggcaaccccacaaacccgttattctttccatgttttcttgagtttcagaggcgaagacacccggaaaaactttactgatcatctctacacagctctcatcaacgctggaattcgaacttttagagatgatgacgaaatccgcaggggagaaaacatagaatctgaactgcaaaagggtattcgagaatccaagatttcactagttgtcttctccaaagattacggttcttcaagatggtgtcttgatgagcttgtcaacattcttgatcgaagaaagaaagagggtcatactgttttgcctgtcttttacactgtgagccccgaggatgtccagaaccaaactggaagttttgctgaagcttttgtgaatcatgaaaagagaggaaatgcagagagtggagataaaagaaaggaatggatggagaagatggacaaatggagagtagctctgaaagaagttgctgaattagaaggaatgtgcttagccaaagaagtagacgggcatgaggcaaaattcatccagaagatcatcaaggagatactcaaaagattgaatcgcacagtacttagtgtaccttcatacacagttggattagagtctcgagtgaaggacattaactcatggttacaggatgaatccagtgaagttggcattgggatgatctgtggacttggtggcgttggaaagactactgttgctaaagtagcttacaactctaattatgacagatttgatgggagttgctttcttgccaatgtcagagaaatctctgagaaacatccaaatggtcaggtttatttgcaaaaacaaatttttgaaagtattttgaaaggcagaaaggaaaaaatatacaatgctgatgaaggaattgtcaaaatgaaagatgctattggcaacaaaaaagtttttattgtatttgatgatgtagatcagctggatgtcttagattcacttattgggacaagggattggttttatccggggagtaaaattctcataacaacaaggtgtgagaaactgttgaagtcctatgagaggcacatgctattcaagataaaggaacttggggttgatgagtctctaaagctcttcagttggtatgcttttgcacaagaccacccattagaagagttcaagatgctttcaacagaagcaatacagcattgtggtgggcttccattagctctttatgatttgggttcgtttctttcagggagagatatggaaatatggagaagcaaattgcagaaattggaagcaatccctcatagcagagttcaaaagaatcttgagataagctacaagtctctagatgatcatgaccagaggttgttcctccttattgcttcattatttgttgggaaggacaaagattatgttatcaaatttttagagaacagcgatttgcacccaacagttggaattcagaacctcattgacagatccctcatcagcattgatgacgaaaacaaagtgatgatgcctccacttattcaggacatgggaaaagaaattattcgtcgagaatcaccagatgatcccgagagattgtgtaaattattgaaccaatgtggtctatcaaattgcttgacagaaaacaatgaaactgatgcagatggagtagacctcccaggcacccatctgccagaagatggtcttgtcccagcacttggccctaatggtgcaaaaagaccatattatcaagattttccagaaatagctgttctaccatacctaggtaattcgttgaaaaggcgctttgtaggacttctttcgacgttccccttatctggtggcctcaaaagattcttcccatga

SEQ ID NO: 18 - DNA, 1821 bp, Solanum candolleanum
  source 1..1821: mol_type = other DNA; note = Rpi-caj1-C419 coding DNA sequence; note (original language) = Rpi-caj1-C419 CDS序列
atggcaaccccacaaacccgttattctttccacgttttcttgagtttcagaggtgaagacacccgaaaaaactttactgatcatctctacacagctctcatcaacgctggaattcgaacttttcgagatgatgacgaaatccgcaggggagaaaacatagaatctgaactgcaaaagggtattcgagaatccaagatttcactagttgtcttctccgaagattacggttcttcaagatggtgtcttgatgagcttgtcaacattcttaatcgaagaaagaaagagggtcatactgttttacctgtcttttacactgtgagccctgaggatgtccagaaccaaactggaagttttgctaaagcttttgtgaatcatgaaaagagaggaaacgcagagagtggagagaaaagaaaggaatggatggagaagatggagaaatggagagtagctctgaaggaagttgctgaattggaaggaatgtgcttagccaaagaagtagacgggcatgaggcaaaattcatccaaaagatcatcaaggagatactcaaaagattgaatcgcacagtacttagtgtaccttcatacacagttggattagagtctcgagtgaaggacattaactcatggttacaggatgaatccagtgaagttggcattgggatgatctgtggacttggtggcattggaaagactactgttgctaaagtagcttacaactctaattatgacagatttgatgggagttgctttcttgcaaatgtcagagaaatctctgagaaacatccaaatggtcaggtttatttgcaaaaacaaatttttgaaagtattttgaaaggcagaaaggacaaaatatacaatgctgatgaaggaattgtcaaaatgaaagatgctattggcaacaaaaaggtttttattgtatttgatgatgtggatcagctggatgtcttggattcacttattgggacaagggattggttttatcctgggagtaaaattctcataacgacaaggtgtgagaaactgttgaagtcctatgagaggcacatgctattcaagataaaggaacttggggttgatgagtctctaaagctcttcagttggtatgcttttgcacaagactacccattagaagagttcaagatgctttcaacagaagcaatacagcattgcggtgggcttccgttagctctttatgatttgggttcgtttctttcagggagaggtatggaaatatggaggagtaaattgcagaaattggaagcaatccctcatagcagagttcaaaagaatcttgagataagctacaagtctctagatgatcatgaccagaggttgttccttcttattgcttcattatttgttgggaaggacaaagattatgttatcaaatttttagagaacagtgatttgcacccaacagttggaattcagaacctcattgacagatctctcatcagcattgatgacgaaaacaaagtgatgatgcctccacttattcaggacatgggaaaagaaattattcgtcgagaatcaccagatgatccggagagattgtgtaaattattgaaccaatgtggtctatcaaattgcttgacagaaaacaatgaaactgatgcagatggagtagacctcccaggcacccatctgccagaagatggtcttgtcccagcacttggtcctaatggtgcaaaaagaccatattatcaagattttccagaaatagctgttctgccatacctaggtaattcgttgaaaaggcgctttgtaggacttctttctacgttccccttatctggtggcctcaaaagattcttcccatga

SEQ ID NO: 19 - DNA, 1806 bp, Solanum cajamarquense
  source 1..1806: mol_type = other DNA; note = Rpi-caj1-C534 promoter sequence; note (original language) = Rpi-caj1-C534 启动子序列
ggttgatctcctttacttgtgctacttatcaatttaagttatttgggaacaaaacaatatgttactgccttactggaatgttcaggtttgtgtattcaatcatccctactatgagtcttgccttgttgccacttgccgctcctacttaactaacacattatactaatagaaacaagggtccttttgattaagggtgacattggagtcttttatttgaggaaatgtgactcaagttttttttatcgggtaaggatgactcttttgaaattagtgttaatgacgctaatttcaaaagcccccaagtgcaccttgtttattagtgttaagggactgataggacatctccttaatgctatgaccttttaaaactgaaatatcacattctcagctcataaccttttctagttgcaccttgattactcggtttatgtggtttgctcctgtaaaaatttcatatggaagatttgaaagatgcagttcactttttgaatgtgtttgatttgctgggttgcaatctcagttgcatattgttttagacagttgctgcaaggtttccatgaatcaaatggcacctaaacattgtttcattcaattctgttgtacaacaacatacccaatttaatctcacaagtggggtctagggagggtggtgtgtacgcagccttgcccctaccttgtcaaggtagagagactatttctgttagacccttggttcaagtgaagccccataacaagtatgggaaggaaatacaatataaagatgtcatgctaaataaaggagaagggaacaacaacaacacataatacggtagaaacatataataataaaattgaagaataagataacaggagagtaataatagcaatattgttatgggaaattggacgacgcttgactacctactaaccttctaccctaatgaacaacatagaaagggaagagatatttaccatatatctttgtctctagatagtccctccactagttcggctaggtagtgatcttcttttgaggcaagagattgagtgggagaaacaacatggtttttgaagcaatatctaattattcatgtgagcatttaatttttgacaaacaagatttagctagatgagattgcttgcccatgccactaatttggaatattttgtatctcattgtactcgtccactgtccaggagtgttgtttctatttggtaaattggcagcagaattcgcaaattgaaaactgacttacgctgcttgttgtgcaggtgaggtggtggtgcaagaactgggatgtctatacagttcagtcgtgtttttttctcagtaatcatcaataagatgcttaacaaacatggacatgttgcctcaatttttttgagacttttgttgtaacaagattaatgagcagtttgctttactatgtattatcctccgttttctataaatctactattccatggctcttccgtcgttctttgcagtttgctcattccactctctccatagcattcatttccagtaggggaagcattaggaaagtattttagtgtggaagtatagaaacctaatcttgctgttcatggatacatgaaaattacaattgagaaaaagaaactctaatactccctaatactttctctgtttcaatttttttggtttttaaactttgcattaagtcgaaaagtaaaatcaaactaacaaattgaactggtgatgcatgccttgtaccatgagcgtttactaaggaataattataaaaaggaagttagaaagaaatttcacagttaagaaagtaccgaccaacttcgcaaatcgcaaca

SEQ ID NO: 20 - DNA, 3186 bp, Solanum cajamarquense
  source 1..3186: mol_type = other DNA; note = Rpi-caj1-C813 promoter sequence; note (original language) = Rpi-caj1-C813启动子序列
tttaaatacgttcatgttgttatagattggagattgtatgatcctatgctaagaaatgtctttggtgatgtttgggtgggtggggtgtggttggtgttcccggaagtgatgtagcctccagtatactcctcttaagcaccatagctatgcaaattgtgttttttctcatctaggtgtaaagattataactacaatgattgaatctagtgccttactttgagttcttttgagtatcttgtcaaaaattatactgtgagttctcttgggtctatacttgtttcattgttagatttctcttatactatgtcttgaaggtatccaatctgtaccttaagcaggaccaccaattttagtattgatcataccacaatcgtctcattaggtacaccagttttcacttgtcctttatctcacctgactgttggatggttgcttttttgtgcaatcagagtttatatgctcaggggtttagatgtgtctctgtcataaaagtgtttgcttcttgtgcaatcagagttgttatgctcaagtggctagatgtgcccctgtcataaaattgaggatgtcttctcctttgcaaagtaatgtctctgcctgtgtctttgatttgattggtgtatgtgtcaaagcatgtccagtgtctgctattacttcctttgagctctctgtattttggtttcctgttgtactctatgcacaattcttaaaataatgcccttttcaatgattttgcatcaatgttgagtcctctggaatttcttccgttgtttgttgttatatattttaataccatgtcttgaaggattctggatacatccttaaagagacaaaaataaggaaaatgccaattgctgtacaaaataatagaacctatccaacttcctttatcaaaaaaataataatagaacctatccaactaccccattaattcactttgtgtcttctgattaactcagtatttgttagttgctgcatgttgcaacaaattactgaagttgttggattttactggaaaacttgggggcttttaaaaacatctgcccaattaaaaaaaaaaaaaaacttgaatcacctctcttaaagaaaagacttaaatgccacccttaattagaggacgttagaaacaagacgagaagagcatatgtcaactaacttctatgtcttattgcacaattacattagataagtgtgggttgatctcctttacttgtgctacttatcaatttaagttatttgggaacaaaacaatatgttactgccttactggaatgttcaggtttgtgtattcaatcatccctactatgagtctggccttgttgccacttgccgctcctacttaactaacacattatactaatagaaacaagggtccttttgattaagggtgacattggagtcttttatttgaggaaatgtgagtcaagtttttttatcgggtaaggattgctcttttgaaattagtgttaatgacgctaattttaaaagcccccaagtgcaccttgtttattagtgttaagggactgataggacatctccttaatgctatgaccttttaaaactgaaatatcacattctcagctcataaccttttctagttgcatcttgtttactcagtttatgtggtctgctcctataaaaattttcatatgaaagatttgaaagatggagtttactttctgaatgtgtttgatttactgggttgcaatctcagttgcatattgttttagacagttgctgcaaggtttccatgaatcaaatggaacctaaacattgtctcattcaattctgttgtacaaaaacatacccaatgtaatctcacaagtagggtctggggagggtggtgtgtactcagctttgcccttaccttgtggaggtagagagactatttccgttaagacccctggctcaagtgaagccccaaaacaagtatgggaaggaaatacacaatataaagatgtcatgctaaatacggaacatataataataaaattgaagaataagataataggaaagtaataatagcaatattgatatgggaaattggatggcgctcgactacctactgaacaacatagaaagggaagagagatttacagtatatctttgtcttcagatagtccctccactagtttggctaggtagtgattgccttttgaggcaggagatcgggagggagaaagaacctggtttcttgaagcaatatctaattattcacgtgagcatttaatttttgacaaacaagatttagctagatgagattgcttgctcatgctgctaatttggaatattttgtatctcattgtactcgtccactgtccagcagtgttgtttctatttggtaaattggcagcagaatttgcaaattgaaaactgacttacgctgcttgttgtgcaggtgaggtggtagtgcaggaactgggatgactatacagttcagtcgtgttttttctcagtaatcatcaataagatacttaacaaaacatggacatgttgcctccatttttttgagacttgtgttgtaacaagattaatgagcagtttgctttactacgtatgttctggttttctataaatctactattccatgggctctcacttctttctttgcagtttgctcattccactttctctccataacattcatttccagtaggggaaatataaggaaaatatttctagtgtggaagtatagaaaccaaatcttgcatttcatggatacatgaaaattacaattgcgaaaaagacactaatatctctttgtttcaatttatttgtttttctaccttgtagtttaagattataagattcaaaaaaaatatttattttcttaaattttgtattaagttgtaaattaaaattaaataaacaaattgtcttgtaccatgagcgtttactaaggaataataattataataaaaaggaaaatgaaggtagaaggaaatttcacagttaagaaagtaccgaccaaattcgcaaatcgcaacacgcaattgccgtaacaaacaaacaaacatacatacattataatacctcgtctcccttcccaccctctacaaaaacattatagttttgactaaaatcctcaattttccatttctgttctctagttttcattgtcaaaatctcaattggatcattatcctctgtctctgcataaactctcatcgttttcttggacttttttca

SEQ ID NO: 21 - DNA, 3181 bp, Solanum sogarandinum
  source 1..3181: mol_type = other DNA; note = Rpi-caj1-C550 promoter sequence; note (original language) = Rpi-caj1-C550启动子序列
aaccaccatagctatgccaattgtgttttttctcatctaggtgtaaagattatactacaatgattgaatctagtgccttcttttgatatgttcatgtcaactttgagttcttttgagtatcttgtcaaaaattaaactgtgagttctctagggtctctacttgtttcattgttagatttctcttatactatgtcttgaaggtatccaatttgtaccttaagcaggaccaccaattttagtattgatcataccacaatcgtctcattaggtacaccagttttcacttgtcttttatctcacctgactgttggatggttgctttttgtgcaatcagagtttatatgctcaggggtttagatatgtccctttcataaaagtgtttgcttcttgtgtaatcagagttgttatgctcaagtggcgaaatgtgcccctgtcataaaattgaggatgtcgtatcctatgcaaagtaatgtctctgcctgtgtctttgatttgattggtgtatgtgtcaaagcgtgtccagtgtgtgctattacttcctttgagctctctgtattttgatttcctgttgtactctatgcacaattcttaaaataatgccttttcaatgattttgcatcaatgttgagtcctctcgaatttcttccactgtttgttgttatatattttaataccatgtcttgaaggattctggatacatccttaaatagacaaaaataaaaaaaatgccaattgctgtacacaataatagaacctattcaacacccccattaattcgctttgtgtcttgtcttctgattaactcagtatttgttagttgctgcatgttgcaacaattatcgaagttgttgcaacaaataactgaagttattggattttactggaaaacttggggggcttttaataacacctacccagtaaaaaaaacttgaataacctctcttaaagaaaagacttaaatgcctcccttaattaaaggacgttagaaacaagacgagaggagcatatgccttctaacttctatatcttattgcacaattacgttagataagtgtgggttgatctcctttacctgtgctacttatcaacttaagttatttgggaacaatatgttactgccttgctggaatgttcaggtttatgtattcaatcatccctactatgagtctggccttgttgccacttgccactcctacttaactaacacattatactaatagaaacaagggtacttttgattaaggcctaagggtgacattggagtcttttatttgaggaaatgtgattcaagtttttttatcgggtagggatgactcttttgaaattagtgttaatgacgctaattttaaaagcccccaagtgcaccttgtttattagtgttaagggaccaataggacatctccttaatgctatgaccttttaaaactgaaacactcacattctcagctcataaccttttctagttgcactttgtttactctgtttatgtggtctgctcctataaaaaaattcatatgaaagatttggaagatgcagtttactttttgaatgtgtttgatttgctgggttgcatattgttttagacagttgctgcaaggtttccatgtcaaatgtgacacctaaacattgtctcattcaattctgttgtacgacaacatacccaatgtaatctcacaagtggggtctgggaagggtggtgtgtactaagccttgcccttaccttgtgaaggtagagagactattttcgttaagacccttggctcaagtgaagccccaaaacaagtatgggaaggaaatacaatataaagatgtcatgctaaaagaaaggagaagggtacaatagcaacaacatatgatacggtggaaacaacatgtaataataaaatggaagaacaagataataggagagtaataatagcaatattgatatgggaaactggacgatgcttggagtattttacagtatatctttgtctccagataagtcccctcactaaaaccaattaatgaacaacatagaaagggaagagagatttacagtatatctttgtctccagataagtcccctcactagttcggctagacagtgatcttcttttgaggcaggagatcgggagggaggaacaacctggtttttgaagcaatatctaattattcaagtgagcatttaatttttgacaaacaagatctagctagatgagattgcttgcccatgctgctaatttggaatattttgtatttcattgtactcgtccactgtccaggagtgttgtttctatttggtaaattggcagcagaatttgcaaattgaaaactgacttacgctgcttgttgtgcaggtgaggtggtagtgcaagaactgggatgtctatacagttcagtcgtgttttttctcagtaatcatcaataagatacttaacaaacatggacatgttgcctcaattttcttgagacttgtgttgtaacaagattaatgagcagtttgctttgctatgtattatcctcggttttgtggttttctatgaatcaactattccatgggctctcccttctttctttgcagtttgctcattccactttctctccatggcattcatttccagtaggggaaacattaggaaaatatttttgtgtggtataaacctagtggaactgacaatataagttcaataatctcgctgttaatggatacataaaaaatacaattgagcaaaagaaactataatactccctctatttcaatttattcgggtttttttttctgtagtttaaaataataagattcaaaaaattcatttacttttttaaacattgtgttaagttgaaaatccaaatcaaacaaataaattgaacttatgagcgtttactaaaggaatatttataaaataaaaaatgaaggtggaaagaaatttcacagttagaaaataccgaccatattcgcaacacgcaattgccttgacacacaaacattataatacctcgtctccctttccaaccccaaacaaaaactcgtcatatttttccccttcacgcgggcctttccattgacttaagtcctcaaagttctaaattttccattttcgttctctagttttcattgtcaaaatctcaattggatcattatcctctttgtctctgcataaactctcagttgggtcatcgttttcttgaacttttttca

SEQ ID NO: 22 - DNA, 3000 bp, Solanum cardiophyllum
  source 1..3000: mol_type = other DNA; note = Rpi-caj1-C509 promoter sequence; note (original language) = Rpi-caj1-C509启动子序列
ttcttaattttatgaaatgggtctcattgatatgctaatgatccgaatgggggtcacttttttttgtttgttgatgaagaagtcttattgatacgaaatagttcatgtgtttaaatacggtcatgttgttatagattggagattgtatgatcatatgctaagaaatgtctttggtgatgtttgggtgggtgggggtgtggttggtgttcctggaagtggtgtagcctccagtatactcctcttaagcaccatagctatgcaaattgtgttttttctcatctaggtgtaaagattataactacaatgattgaatctagtgccttcttttgatatgttcatatcaactttgagttcttatgagtatcttgtcaaaaattatactgtgagttttcttgggtctctacttgtattgatcataccacaatcgtcttattaggtacaccagttttcacttgtcctttatctcacctgactgttggatggttgctttttgtgcaatcagagtttatatgctcagggttttagatgtgtctctgtcataaaagtgtttgcttcttgtgcaatcagagttgttatgctcaagtggctaggtgtacccctgtcataaaattgaggatgtcttctcctttgcaaagtaatgcctctgcctgtgtctttgatttgattggtgtatgtgtcaaagcgtgtccagtgtctgctattacttcctttgagctctctgtatttggtttcctgttgtactctatgcacaattcttaaaataatgccttttcaatgattttgcatcaatgttgagtcctctggaatttcttccgttgtttgttgtaatatattttaataccatgtcttgaaggattctggatacatccttgaagggacaaaaataaggaaaatgccaattgctgtacaaaataatagaacctatccaactacccatttaattcgctttgtgtcttctgataactcagtattttttagttgctgcatgttgcaacaaattactgaagttgttggattttactggaaaacttgggggcttttaaaaacacctgcccaaaaaaaaaacttgaatcacctctcttaaagaaatgacttaaatgccacccttaattaaaggacgttagaaacaagacgagaagagcatatgcctactaacttctatgtcttattgcacaattacattagataagtgtgggttgatctcctttacttgtgctacttatcaatttaagttatttgggaacaaaacaatatgttactgccttactggaatgttcaggtttgtgtattcaatcatccctactatgagtcttgccttgttgccacttgccgctcctacttaactaacacattatactaatagaaacaagggtccttttgattaagggtgacattggagtcttttatttgaggaaatgtgactcaagttttttttatcgggtaaggatgactcttttgaaattagtgttaatgacgctaatttcaaaagcccccaagtgcaccttgtttattagtgttaagggactgataggacatctccttaatgctatgaccttttaaaactgaaatatcacattctcagctcataaccttttctagttgcaccttgattactcggtttatgtggtttgctcctgtaaaaatttcatatggaagatttgaaagatgcagttcactttttgaatgtgtttgatttgctgggttgcaatctcagttgcatattgttttagacagttgctgcaaggtttccatgaatcaaatggcacctaaacattgtttcattcaattctgttgtacaacaacatacccaatttaatctcacaagtggggtctagggagggtggtgtgtacgcagccttgcccctaccttgtcaaggtagagagactatttctgttagacccttggttcaagtgaagccccataacaagtatgggaaggaaatacaatataaagatgtcatgctaaataaaggagaagggaacaacaacaacacataatacggtagaaacatataataataaaattgaagaataagataacaggagagtaataatagcaatattgttatgggaaattggacgacgcttgactacctactaaccttctaccctaatgaacaacatagaaagggaagagatatttaccatatatctttgtctctagatagtccctccactagttcggctaggtagtgatcttcttttgaggcaagagattgagtgggagaaacaacatggtttttgaagcaatatctaattattcatgtgagcatttaatttttgacaaacaagatttagctagatgagattgcttgcccatgccactaatttggaatattttgtatctcattgtactcgtccactgtccaggagtgttgtttctatttggtaaattggcagcagaattcgcaaattgaaaactgacttacgctgcttgttgtgcaggtgaggtggtggtgcaagaactgggatgtctatacagttcagtcgtgtttttttctcagtaatcatcaataagatgcttaacaaacatggacatgttgcctcaatttttttgagacttttgttgtaacaagattaatgagcagtttgctttactatgtattatcctccgttttctataaatctactattccatggctcttccgtcgttctttgcagtttgctcattccactctctccatagcattcatttccagtaggggaagcattaggaaagtattttagtgtggaagtatagaaacctaatcttgctgttcatggatacatgaaaattacaattgagaaaaagaaactctaatactccctaatactttctctgtttcaatttttttggtttttaaactttgcattaagtcgaaaagtaaaatcaaactaacaaattgaactggtgatgcatgccttgtaccatgagcgtttactaaggaataattataaaaaggaagttagaaagaaatttcacagttaagaaagtaccgaccaacttcgcaaatcgcaaca

SEQ ID NO: 23 - DNA, 3124 bp, Solanum piurae
  source 1..3124: mol_type = other DNA; note = Rpi-caj1-C450 promoter sequence; note (original language) = Rpi-caj1-C450启动子序列
catgtgtttaaatacgttcatgttgttatcgattggagattgtatgatcctatgctaagaaatgtctttggtgatgtttgggagggtgggggtgtggttggtgttcccggaagtgatgtagcctccagtatactcctcttaagcaccatagctatgcaaattgcgttttttctcatctaggtgtaaagattataactacaatgattgaatctagtgccttactttgagttcttttgagtatcttgtcaaaaattatactgtgagttcttttgggtctctacttgtttcattgttagatatctcttatactatgtcttgaaggtatccaatctgtaccttaagcaggaccaccaattttagtattgatcataccacaatcgtctcattaggtacaccagttttcacttgtcctttatctcacctgactgttggatggttgctttttgtgcaatcagagtttatatgctcaggggtttagatgtgtctctgtcataaaagtgtttgcttcttgtgcaatcagagttgttatgctcaagtggctagatgtgcccctgtcataaaattgaggatgtcttctcctttgcaaagtaatgtctctgcctgtgtctttgatttgattggtgtatgtgtcaaagcgtgtccagtgtgtgctattacttcctttgagctctctgtattttggtttcctgttgtactctatgcacaattcttaaaataatgccttttcaatgattttgcatcaatgttgagtcctctggaatttctcccgttgtttgttgttatatattttaataccatgtcttgaagggttctggatacatccttaaagagacaaaaagaaggaaaatgccaattgctgtacaaaataatagaacctatccaactaccccattaattcgctttgtgtcttctgattaactcagtatttgttagttgctgcatgttgcaacaaattactgaagttgttggattttactggaaaactttggggcttttaaaaacacctgcccaattaaaaaaaaaacttgaatcacctctcttaaagaaaagacttaaatgccacccttaattaaaggacgttagaaacaagacgagaagagcatgtgcctactaatttctatgtcttattgcacaattacattagataagtgtgggttgatctcctttacttgtgctacttatcaatttaagttatttgggaacaaaacaatatgttactgccttactggaatgttcaggtttgtgtattcaatcatccctactatgagtgtggccttgttgccacttgccgctcctacttaactaacgcattatactaatagaaacaagggtccttttgattaagggtgacattggagtcttttatttgaggaaatgtgactcaagtttttttatcgggtaaggatgactcttgagaaattagtgttaatgacgctaattttaaaagcccccaagtgcaccttgtttattagtgttaagggactgataggacatctccttaatgctatgaccttttaaaactgaaatatcacattctcagctcataaccttttctagttgcatcttgtttatgtggtctgctcctataaaaaatttcatatgaaggatttgaaagatgcagtttactttctgaatgtgtttgatttactgggttgcaatctcagttgcatattgttttagacagttgctgcaaggtttccatgaatcaaatggcacctaaacattgtctcattcaattctgttgtacaaaaacatacccaatgtaatctcacaagtagggtctggggagggtggtgtgtactcagctttgcccttaccttgtgaaggtagagagactatttctgttaagacccctagctcaagtgaagccccaaaacaagtatgggaaggaaatacaatataaagatgtcatgctaaatacggtggaaacatataataataaaattgaagaataagataataggagagtaataatagcaatattgatatgggaaattggatggcgctcgactacctactgaacaacatagaaagggaagagagatttacaggatatctttgtctccagatagtccctccactagttcggctaggtagtgattgtcttttgaggcaggagatcgggagggagaaagaacctggtttcttgaagcaatatctaattattcacgtgagcatttaatttttgacaaacaagatttagctagataagattgcttgctcatgctgctaatttggaatattttgtatctcatcgtacttgtccactgtccagcagtgttgtttctatttggtaaattggcagcagaatttgcaaattgaaaactgacttacgctgcttgttgtgcaggtgaggtggtagtgcaagaactgggatgactatacagttcagtcgtgttttttctcagtaatcatcaataagatacttaacaaacatggtcatgttgcctcaatttttttgagacttgtgttgtaacaagattaatgagcagtttgctttactatgtatgttctggttttctataatctactattccatgggctctcccttctttctttgcagtttgctcattccactttctctccatagcattcatttccagtaggggaaacataaggaaaatatttttagtgtgcaagtatagaaacctaatcttgctgttcatggatacatgaaaattacaattgagaaaaagaaactctaatactccctctgtttcaatttatttgtttttctaccttatagtttaagatcataagattcaaaaaaattatttattttcttaaatttcatattaaatcgtaaattataatcaaacaaacaaattgtctgtgtttactaaggaataattataaaaaggaaaatgaaggtagaaagaaatttcacagttagaaagtaccgaccaaattcgcaaatcgcaacacgcaattgccttaaacaaacaaacattataataactcgtctcccttcccacccctacaaaaacattatagtattgacttaaatcctcaattttccatttctgttctctagttttcattgtcaaaatctcaattggatcattatcctctttgtctctgcataaactctcagttgggtgatcgttttcttggacttttttca

SEQ ID NO: 24 - DNA, 3184 bp, Solanum candolleanum
  source 1..3184: mol_type = other DNA; note = Rpi-caj1-C419 promoter sequence; note (original language) = Rpi-caj1-C419启动子序列
gtagcctccactatactcctcttaagcaccgtagctatgccaattgtgttttttctcatctaggtgtaaagattatactacaaggattgaatctagtgccttcttttgatatgttcatgtcaactgtgagttcttttgagtatcttgtcaaaaattaaactgtgagttctctagggtctctacttgtttcattgttagatttctcttataccatgtcttgaaggtatccaatttgtaccttaagcaggaccaccaattttagtattgatcataccacaatcgtctcattaggtacaccagttttcacttgtcctttatctcacctgactgttggatggttgctttttgtgcaatcagagtttatatgctcaggggtttagatatgtccctttcataaaagtgtttgcttcttgtgtaatcagagttgttatgctcaagtggcgaaatgtgcccctgtcataaaattgaggatgtcgtctcctatgcaaagtaatgtctctgcctgtgtctttgatttgattggtgtatgtgtcaaagcgtgtccagtgtgtgctattacttcctttgggctctctgtatttaaatttcctgttgtactctatgcacaattcttaaaataatgccttttcaatgattttgcatcaatgttgagtcctctcgaatttcttccactgtttgttgttatatattttaataccatgtcttgaaggattctggatacatccttaaagagacaaaaataaaaaaaatgccaattgctgtacacaataatagaacctatccaacacccccattaattcgctttgtgtcttgtcttctgattaactcagtatttgttagttgctgcatgacaattatcgaagttgttgcaacaaataactgaagttattggattttactggaaagcttggggggcttttaataacacctgcccagttaaaaaaacttgaataacctctcgtaaagagaagacttaaatgcctcccttaattaaaggacgttagaaacaagacgagaggagcatatgccttctaacttctatatcttattgcacaattacgttagataagtgtgggttgatctcctttacctgtgctacttatcaacttgagttatttggggttactgccttactggaatgttcaggtttatgtattcaatcatccctactatgagtctggccttgttgccacttgccactcctacttaactgactcattatactaatagaaacaaggacccttttgattaagggtgacattggagtcttttatgtgaggaaatgtgactcaagtttttttattgggtagggatgactcttttgaaattagtgttaatgacacactaatttaaaagcccccacaagtgcaccttgtttattagtgttaaggggccgataagacatctcctttatgctatgaccttttaaactgaaatactcacattctcagctcataaccttttctagttgcatcttgtttactcggtttatgtggtctgctcctataaaaattttcatatgaaagatttgaaagatgcagtttactttctgaatgtgtttgatttagtgggttgcaatctcagttgcatattgttttagacagttgcatattgttttagacagttgcatattgttttagacagttgctgcaacgtttccatttatcaaatggcacctaaacattgtttcattcaattctgttgtacaacaacatacccaatgtaatctcacaagtggggttagggagggtggtgcttacgcaaccttgcccctaccttatcaaggtagagaaactatttccgttagacccttggctcaagtgatgccccataacaagtatgggaaggaaatacaatataagatgtcatgctaaataaaggagaagttaacaacaacatataatacggtggaaacatataataataaaattgaagaaaaagataacaggagagtaataatagcaatattgttatgggaaactggatgacgctcgactacctactaaccttctaccctaatgaacaacatagaaagggaagagagatttaccatatatctttgtctccagatagtccctccactagttcggctaggtagtgatcttcttttgaggcaggagatcgggagggagaaagaacctggttttttgaagcaatatctaattattcacgtgagcatttaatttttgacaaacaagatttagctagatgagattgcttgcccatgctgctaatttggaatattttgtatctcctcgtactcgtccacggtctagcagtgttggttgtatttggtaaattggcagcagaatttgcaaattgaaaactgacttacgctgcttgttgtgcaggtgaggtggtagtttaagaactgggatgactatacagttcagtcgtgttttttctcagtaatcatcaataagatacttaacaaacatggacatgttgcctcaatttttttgagacttgtgttgtaacaagattaatgagcagtttgctttactatgtattgtcctcgattttgtggttttctaataaaattactattccatcggctctctcttctttctctccatagcattcatttccagtaggggaaacattaggaaaatatttgtgtggaagtatttatgtcatattctgggtataaacctagtggaactgacaatataagttcaataatcttgctgttaatggatacataaaaaatacaattgagcaaaagaaactataatactccctctgtttcaatttatttgggtttttttttcttctgtagtttaaaataataagattcatttacttttttaaacattgtgttaagtcgaaaatccaaatcaaacaaataaattgaacttatgagcgtttactaaaggaatgtttataaaagaaaaaatgtaggtggaaagaaatttcacagttagaaaataccgaccatattcgcaacacgcaattgccttaacacacaaacattataatacctcgtctccctttccaaccccaaacaaaaactcgtcatttttttccccttcacgcgggcctttccattgacttaagtcctcaaagttctaaattttccattttcgttctctagttttcatcttcaaaatctcaattggatcattatcctctttgtctctgcataaactctcagttgggtcatccttttcttgaacttttttca

SEQ ID NO: 25 - DNA, 44 bp, synthetic construct
  source 1..44: mol_type = other DNA; note = Rpi-caj1-C534 forward primer sequence; note (original language) = Rpi-caj1-C534 上游引物序列
tcgacggtaccgcgggcccatggcaaccccacaaacccgttatt

SEQ ID NO: 26 - DNA, 42 bp, synthetic construct
  source 1..42: mol_type = other DNA; note = Rpi-caj1-C534 reverse primer sequence; note (original language) = Rpi-caj1-C534 下游引物序列
tagactaggtggatcccctaccaagacaagcttaacatgaat

SEQ ID NO: 27 - DNA, 45 bp, synthetic construct
  source 1..45: mol_type = other DNA; note = Rpi-caj1-C534 forward primer sequence containing promoter; note (original language) = 包含启动子的Rpi-caj1-C534 上游引物序列
gttaattaagaattcaccggggttgatctcctttacttgtgctac

SEQ ID NO: 28 - DNA, 46 bp, synthetic construct
  source 1..46: mol_type = other DNA; note = Rpi-caj1-C534 reverse primer sequence containing promoter; note (original language) = 包含启动子的Rpi-caj1-C534 下游引物序列
tagactaggtggatccctcatgggaagaatctcttgaggctaccag

SEQ ID NO: 29 - DNA, 46 bp, synthetic construct
  source 1..46: mol_type = other DNA; note = Rpi-caj1-C813 forward primer sequence; note (original language) = Rpi-caj1-C813上游引物序列
cgaattctgcagtcgaccccatggcaaccccacaaacccgttattc

SEQ ID NO: 30 - DNA, 46 bp, synthetic construct
  source 1..46: mol_type = other DNA; note = Rpi-caj1-C813 reverse primer sequence; note (original language) = Rpi-caj1-C813下游引物序列
tacaagaaagctgggtcccctgggaagaatctcttgaggctaccag

SEQ ID NO: 31 - DNA, 46 bp, synthetic construct; identical to SEQ ID NO: 29
  source 1..46: mol_type = other DNA; note = Rpi-caj1-C550 forward primer sequence; note (original language) = Rpi-caj1-C550上游引物序列

SEQ ID NO: 32 - DNA, 46 bp, synthetic construct
  source 1..46: mol_type = other DNA; note = Rpi-caj1-C550 reverse primer sequence; note (original language) = Rpi-caj1-C550下游引物序列
tacaagaaagctgggtcccctgggaagaatcttttgaggccaccag

SEQ ID NO: 33 - DNA, 43 bp, synthetic construct
  source 1..43: mol_type = other DNA; note = Rpi-caj1-C509 forward primer sequence; note (original language) = Rpi-caj1-C509上游引物序列
cgaattctgcagtcgacccccgcaattgccttaacaaacaaac

SEQ ID NO: 34 - DNA, 46 bp, synthetic construct; identical to SEQ ID NO: 32
  source 1..46: mol_type = other DNA; note = Rpi-caj1-C509 reverse primer sequence; note (original language) = Rpi-caj1-C509下游引物序列

SEQ ID NO: 35 - DNA, 46 bp, synthetic construct; identical to SEQ ID NO: 29
  source 1..46: mol_type = other DNA; note = Rpi-caj1-C450 forward primer sequence; note (original language) = Rpi-caj1-C450上游引物序列

SEQ ID NO: 36 - DNA, 46 bp, synthetic construct; identical to SEQ ID NO: 32
  source 1..46: mol_type = other DNA; note = Rpi-caj1-C450 reverse primer sequence; note (original language) = Rpi-caj1-C450下游引物序列

SEQ ID NO: 37 - DNA, 40 bp, synthetic construct
  source 1..40: mol_type = other DNA; note = Rpi-caj1-C419 forward primer sequence; note (original language) = Rpi-caj1-C419上游引物序列
cgaattctgcagtcgaccccatggcaaccccacaaacccg

SEQ ID NO: 38 - DNA, 43 bp, synthetic construct
  source 1..43: mol_type = other DNA; note = Rpi-caj1-C419 reverse primer sequence; note (original language) = Rpi-caj1-C419下游引物序列
tacaagaaagctgggtcccctgggaagaatcttttgaggccac